European Patent Specification EP 3 570 838 B1, published June 5, 2024. Title: Substituted 3-Dialkylaminomethyl-Piperidin-4-yl-Benzamides and Methods of Making and Using Same. Applicant: Mebias Discovery LLC Tounge, Brett A Bayoumi, Shariff Kuo, Lawrence C Dax, Scott L. The sequence listing filed with the application follows.

SEQUENCE LISTING (1 sequence)

SEQ ID NO: 1 - protein, 4 aa, Artificial Sequence
  Chemically synthesized
  MOD_RES (2)..(2): D-Ala
  MOD_RES (4)..(4): Tyr methylated on alpha-NH2 and amidated with -NHCH2CH2OH on C-terminus
YXGX